European Patent Application EP 4 678 752 A1, published January 14, 2026. Title: YARROWIA SP. MICROORGANISM FOR PRODUCING RETINOL WITH REDUCED ABC3 PROTEIN ACTIVITY AND RETINOL PRODUCTION METHOD USING SAME. Applicant: CJ CHEILJEDANG CORPORATION. Application KR. The sequence listing filed with the application follows.

SEQUENCE LISTING (46 sequences)

SEQ ID NO: 1 - protein, 1485 aa, Yarrowia lipolytica
MTDPVPITQDPTIYSSQQDAEIRSLAESIHSQHSNNSNNSTELTNPYVDTSDPELDPWSGQFNSRKWSRTILGLKRRYGTSKEITAGVSFKNLGAYGYGGGADYQKTVANAVLGLEGVVRTLFHLEKKEDKVQILSDFNGVLWPGETCVVLGRPGSGCTTLLKSIACETYGFQLDKETEWNYQGIPRKIMQKTCRGEIVYNAEVDVHFPHLTVGDTLMFASLARTPQNRFDGVTREQYAKHTRDVTMASLGLSHTLDTKVGNDFVRGVSGGERKRVSIAESIVCGSPLQCWDNSTRGLDAATATEFLRWLRHSAELTGASMFVSLYQASQEAYELFDKVTVLYEGQQIYFGPGEQAKQYFEEMGFECPHRQTTGDFLTSITSPAERIVAPGFEGKTPRTASEFAERWRQSQAYANLQEEIERFNTEFPVGGNRVADIMELKQEKQSDHIKVSSPYTISIPMQVKLCLTRGFQRLRGDLSMALTTVLGNFVVALILSSMFYNMPEDTSSFFSRGALLFFAMLMNAMSSVLEIIVLYELRPIVEKHQRYAMYHPFCEALASIICDFPTKFLTMLCVNVTLYFMSNLRREAGPFFIFFLFTLLCVLAMSMIFRTIAAVTKTLQQALAPAAVIILALIIYTGFTLPISYMRGWARWINYIDPIAYGFEAVMVNEFRNREFPCALFIPQQSTYDQLGSPYQGCMAVGAKPGERFVNGDRYLEMAFDYSQAHLWRNLGIMFGFILFFAFTYLTAVEFIQSAKSKGEVLVFLRSSLKQRKKRAHLMDVEANAEKVGAAQDREILVQQEEGQQEETSSCTPSDSTPKDIFQWKDVCYDIKVKGGEKRLLDNVDGWVKPGTLTALMGCSGAGKTTLLDVLADRKATGVITGDMRVNGQKRDASFQRKTGYVQQQDLHTATSTVREALEFSALLRQPSNVPKAEKIAYVDEVIDILEMQAYADAVVGVPGEGLNVEQRKRLTIGVELAAKPELLLFLDEPTSGLDSQTAWSIICLLKKLANRGQAILCTIHQPSAILFQEFDRLLFMTLGGKTVYYGDIGANSSALINYFESKGADPCPEEANPAEWMLAAIGAAPGSIAKHDWAVVWNESEERARERDLLDKMAEELAAQSTHDEKNELVTSKSVGSSQTSSSSYSAKSQYATSQATQLYYLTKRLWTYYWRSPRYIWSKLLMSIASALFIGFSYYKASQDIQGLQNQMFAFFMLFLIFVIIMVQILPHFVAQRELYEARERSSMAYSWQAFMGSNILVELPWQTLVAVLVFFCFYYPIGLQNNATGHLGERGALFFLLLWSFYVYNSTFAHMMGAAFENKENAATIGYLLFALCLIFCGVLATKEDMPHFWIFMYRVSPLTYLISGLLSAGVGETRVECTDNELVLFKPMNGTNCGKYMHPFMEGLGHTDMPMGYLVDPSATDMCGYCPISNTNGYLDQIDVKYSQRWRNYGILFAYPAFNVFMAFAFYYIFRVPKKSRKQKA

SEQ ID NO: 2 - DNA, 4458 bp, Yarrowia lipolytica
  source 1..4458: mol_type = genomic DNA
atgacagatcctgtaccgatcacgcaggatccgaccatctactcgagtcagcaagacgccgagatccggtcgttggccgagtccattcactcacagcattccaacaattccaacaactccacagagcttaccaacccgtatgtcgatacctctgatccagagctcgatccctggagcggccagttcaacagtcggaaatggtccaggacaattttgggtctgaaacgacgatatggcacctccaaggagatcactgccggcgtgtctttcaaaaacctcggcgcctatggatatggtggaggagccgattaccagaagactgtggccaacgcagtgctaggtctggagggcgttgtgcgtactcttttccatctggagaagaaggaagataaggtgcagattctctctgacttcaacggtgtgctatggcctggggagacctgtgttgtccttggacgacctggttctggatgtacgactctgctaaagagtattgcttgcgagacgtacggatttcagctcgacaaagagactgaatggaattatcagggcattccccgaaaaatcatgcagaaaacctgccgtggtgaaatcgtgtacaacgcagaagttgacgtgcatttccctcatctcacagtcggagacaccctcatgttcgcctctctggcccgaactccccagaaccgattcgatggagtcacccgagaacagtatgcaaagcatactcgagacgtgaccatggcctctctgggtctgtctcacactctcgacaccaaggttggaaatgactttgtgcgaggtgtttctggaggagagcgaaagcgagtctctatcgccgagagtattgtctgtggatcgcctctgcagtgctgggacaacagtactcgaggtctcgatgctgctactgccaccgagtttctgcgatggctgcgtcactcagccgagctcactggcgcctccatgtttgtgtctctctaccaggcctcccaggaagcctacgaactctttgacaaggtgaccgttctctacgagggtcagcagatctactttggtcccggtgagcaagccaagcaatactttgaagagatgggattcgaatgtcctcatcgacagacaaccggagacttcctcacatctattacctctcctgcagagcgaattgtcgctcctggctttgaggggaagacccctcgaactgcatccgaatttgctgagcgatggagacagtcccaggcctatgccaaccttcaggaggagattgagcgattcaacaccgagtttcccgtgggaggaaaccgagttgccgatatcatggagctcaaacaggagaagcagagtgaccatatcaaggtgtcttctccctacacaatctccatccccatgcaggtcaagctgtgcttgacccgaggcttccaaagactcagaggcgatctcagtatggctctgaccactgtcttgggtaactttgtcgttgctctcattctctcgtctatgttctacaacatgcccgaagacacatcgtccttcttttcccgaggagctcttctattctttgccatgttgatgaacgccatgtcttctgttcttgaaatcattgtcctttacgaacttcgtcccattgtggaaaagcaccagagatacgccatgtaccaccccttctgtgaagcgttagcgtcaattatctgcgacttccccaccaaattcctcaccatgctttgtgtcaacgtgactctttacttcatgtccaacctgcgacgagaagccggtccttttttcatcttcttcctcttcacactcctatgtgttttggccatgagtatgattttccgaaccattgcagctgtcaccaaaactcttcagcaggcccttgctcccgcagctgtcattattctcgcccttatcatctacacaggcttcactctccccattagctacatgcgaggatgggcacggtggatcaactatattgacccgattgcctacggctttgaagcggtcatggtcaacgagttccgaaacagagaattcccttgtgcccttttcatcccacagcagtccacatacgaccagctgggatctccttaccagggctgtatggccgttggagcaaagcctggagagcgttttgtcaacggagaccggtacttggaaatggcctttgattactcgcaggctcacttgtggcgaaacctgggtatcatgtttggcttcattctcttctttgcgttcacctacctgactgccgtcgagttcatccagtctgccaaatccaagggtgaggttctggtgttcctgcgatcttctctcaagcagcgaaagaagcgagctcatctgatggatgtcgaggccaatgctgagaaggttggtgcagctcaggatagagagattcttgttcagcaggaggagggtcagcaggaagagacttcctcgtgtaccccctccgattctacccccaaggatatcttccaatggaaggatgtgtgctacgacatcaaggtaaagggcggagaaaagagactactggataacgtggacggatgggtcaagccaggtactctaacagccctcatgggctgctctggagccggtaaaaccactcttctggatgttctggctgaccgaaaggccactggtgtgattactggagacatgcgagtcaacggacagaagcgggacgcctctttccagagaaagacaggttacgtgcaacagcaggatctccatactgctacttccaccgttcgtgaagctctcgagttttctgctcttctgcgacaaccttccaatgtgcccaaggccgagaagattgcctatgttgacgaagtcattgatattctggagatgcaggcctatgctgatgctgttgtcggtgtccccggtgaaggtctcaacgttgagcagcgaaagcgactaactatcggtgtagagcttgctgccaagcctgaactcctgctgttccttgatgagcccacttccggtcttgactcccagactgcctggtcaatcatctgtctgctgaagaaactagccaaccgaggccaggctattctgtgtactattcatcagccctctgccattctcttccaagagtttgaccgtcttctgttcatgactctgggaggtaagactgtttactacggagatatcggagccaactcgtctgcattgatcaactacttcgagtccaagggtgccgatccttgtcctgaagaggctaaccctgctgaatggatgcttgctgctattggagctgcccccggaagtattgccaagcacgattgggctgtagtctggaacgagagtgaagagcgagcccgagagcgagatctgcttgataagatggccgaggagcttgctgctcagagtactcatgatgagaagaacgagctggtaacctccaagagcgtcggaagctcccagacctcctcttcgtcatactctgccaagtcccagtacgccacatctcaggctactcagctgtactaccttaccaagcgactgtggacctactactggcgatctccccgatatatctggtccaagctactcatgtccattgcctctgccctgtttattggtttctcttactacaaggcgtcacaagacatccagggtctccagaaccagatgtttgccttcttcatgcttttcctcatcttcgtcatcatcatggtccagattctgccccatttcgtggcccagcgagaactctacgaggcgcgagagcgatcttccatggcttattcgtggcaggctttcatgggctctaacatcctcgtcgagcttccctggcagactctggtggcagttcttgtcttcttctgcttttactaccccattggcctgcagaataacgctactggccatcttggcgaacgaggagccctcttcttcctcttgctctggtccttctacgtctacaactccacttttgctcacatgatgggagccgccttcgagaacaaggagaacgcagccaccattggttacctgctctttgctctctgtctgatcttctgtggtgttctggccaccaaggaggacatgccccacttctggatcttcatgtaccgagtgtctccgctgacttacctcatttccggcctcctcagtgcaggtgtcggagagaccagagttgagtgcaccgataacgagcttgtcctgttcaagcccatgaacggaaccaactgtggaaaatacatgcatccgttcatggagggtcttggacacacagacatgcccatgggctatctggtcgacccatccgccaccgacatgtgtggatattgccccatttccaacaccaacggctaccttgaccagattgatgtcaagtacagtcagcgatggcgaaactatggcattctgtttgcctaccctgccttcaacgtctttatggcttttgctttctactatatcttccgagtccccaaaaagtctcgaaagcagaaggcctag

SEQ ID NO: 3 - DNA, 406 bp, synthetic construct
  source 1..406: mol_type = other DNA
agagaccgggttggcggcgcatttgtgtcccaaaaaacagccccaattgccccaattgaccccaaattgacccagtagcgggcccaaccccggcgagagcccccttctccccacatatcaaacctcccccggttcccacacttgccgttaagggcgtagggtactgcagtctggaatctacgcttgttcagactttgtactagtttctttgtctggccatccgggtaacccatgccggacgcaaaatagactactgaaaatttttttgctttgtggttgggactttagccaagggtataaaagaccaccgtccccgaattacctttcctcttcttttctctctctccttgtcaactcacacccgaaatcgttaagcatttccttctgagtataagaatcattcaaa

SEQ ID NO: 4 - DNA, 1533 bp, synthetic construct
  source 1..1533: mol_type = other DNA
tgcctcctgtctgactcgtcattgccgcctttggagtacgactccaactatgagtgtgcttggatcactttgacgatacattcttcgttggaggctgtgggtctgacagctgcgttttcggcgcggttggccgacaacaatatcagctgcaacgtcattgctggctttcatcatgatcacatttttgtcggcaaaggcgacgcccagagagccattgacgttctttctaatttggaccgatagccgtatagtccagtctatctataagttcaactaactcgtaactattaccataacatatacttcactgccccagataaggttccgataaaaagttctgcagactaaatttatttcagtctcctcttcaccaccaaaatgccctcctacgaagctcgagctaacgtccacaagtccgcctttgccgctcgagtgctcaagctcgtggcagccaagaaaaccaacctgtgtgcttctctggatgttaccaccaccaaggagctcattgagcttgccgataaggtcggaccttatgtgtgcatgatcaagacccatatcgacatcattgacgacttcacctacgccggcactgtgctccccctcaaggaacttgctcttaagcacggtttcttcctgttcgaggacagaaagttcgcagatattggcaacactgtcaagcaccagtacaagaacggtgtctaccgaatcgccgagtggtccgatatcaccaacgcccacggtgtacccggaaccggaatcattgctggcctgcgagctggtgccgaggaaactgtctctgaacagaagaaggaggacgtctctgactacgagaactcccagtacaaggagttcctggtcccctctcccaacgagaagctggccagaggtctgctcatgctggccgagctgtcttgcaagggctctctggccactggcgagtactccaagcagaccattgagcttgcccgatccgaccccgagtttgtggttggcttcattgcccagaaccgacctaagggcgactctgaggactggcttattctgacccccggggtgggtcttgacgacaagggagacgctctcggacagcagtaccgaactgttgaggatgtcatgtctaccggaacggatatcataattgtcggccgaggtctgtacggccagaaccgagatcctattgaggaggccaagcgataccagaaggctggctgggaggcttaccagaagattaactgttagaggttagactatggatatgtcatttaactgtgtatatagagagcgtgcaagtatggagcgcttgttcagcttgtatgatggtcagacgacctgtctgatcgagtatgtatgatactgcacaacctgtgtatccgcatgatctgtccaatggggcatgttgttgtgtttctcgatacggagatgctgggtacaagtagctaatacgattgaactacttatacttatatgaggcttgaagaaagctgacttgtgtatgacttattctcaactacatccccagtcacaataccacca

SEQ ID NO: 5 - DNA, 24 bp, synthetic construct
  source 1..24: mol_type = other DNA
gtccacttctacagcaacattatg

SEQ ID NO: 6 - DNA, 46 bp, synthetic construct
  source 1..46: mol_type = other DNA
gacgagtcagacaggaggcaggtacgatagtaaagtctgttgatac

SEQ ID NO: 7 - DNA, 46 bp, synthetic construct
  source 1..46: mol_type = other DNA
gtatcaacagactttactatcgtacctgcctcctgtctgactcgtc

SEQ ID NO: 8 - DNA, 40 bp, synthetic construct
  source 1..40: mol_type = other DNA
aatggttggatgagggtggatggtggtattgtgactgggg

SEQ ID NO: 9 - DNA, 40 bp, synthetic construct
  source 1..40: mol_type = other DNA
ccccagtcacaataccaccatccaccctcatccaaccatt

SEQ ID NO: 10 - DNA, 43 bp, synthetic construct
  source 1..43: mol_type = other DNA
gccacagttttgacgtaataagcggtacgatagtaaagtctgt

SEQ ID NO: 11 - DNA, 43 bp, synthetic construct
  source 1..43: mol_type = other DNA
acagactttactatcgtaccgcttattacgtcaaaactgtggc

SEQ ID NO: 12 - DNA, 22 bp, synthetic construct
  source 1..22: mol_type = other DNA
gagatgaactgtccaaatcgag

SEQ ID NO: 13 - DNA, 20 bp, synthetic construct
  source 1..20: mol_type = other DNA
gtatgtgcctggatcgtacc

SEQ ID NO: 14 - DNA, 20 bp, synthetic construct
  source 1..20: mol_type = other DNA
caacaactcgggatccactc

SEQ ID NO: 15 - DNA, 24 bp, synthetic construct
  source 1..24: mol_type = other DNA
gtccacttctacagcaacattatg

SEQ ID NO: 16 - DNA, 45 bp, synthetic construct
  source 1..45: mol_type = other DNA
cgccgccaacccggtctctggtacgatagtaaagtctgttgatac

SEQ ID NO: 17 - DNA, 45 bp, synthetic construct
  source 1..45: mol_type = other DNA
gtatcaacagactttactatcgtaccagagaccgggttggcggcg

SEQ ID NO: 18 - DNA, 40 bp, synthetic construct
  source 1..40: mol_type = other DNA
gacgagtcagacaggaggcatttgaatgattcttatactc

SEQ ID NO: 19 - DNA, 40 bp, synthetic construct
  source 1..40: mol_type = other DNA
gagtataagaatcattcaaatgcctcctgtctgactcgtc

SEQ ID NO: 20 - DNA, 40 bp, synthetic construct
  source 1..40: mol_type = other DNA
gcgccgccaacccggtctcttggtggtattgtgactgggg

SEQ ID NO: 21 - DNA, 40 bp, synthetic construct
  source 1..40: mol_type = other DNA
ccccagtcacaataccaccaagagaccgggttggcggcgc

SEQ ID NO: 22 - DNA, 49 bp, synthetic construct
  source 1..49: mol_type = other DNA
gtgatcggtacaggatctgtcattttgaatgattcttatactcagaagg

SEQ ID NO: 23 - DNA, 49 bp, synthetic construct
  source 1..49: mol_type = other DNA
ccttctgagtataagaatcattcaaaatgacagatcctgtaccgatcac

SEQ ID NO: 24 - DNA, 21 bp, synthetic construct
  source 1..21: mol_type = other DNA
cacgtctcgagtatgctttgc

SEQ ID NO: 25 - DNA, 20 bp, synthetic construct
  source 1..20: mol_type = other DNA
gtatgtgcctggatcgtacc

SEQ ID NO: 26 - DNA, 22 bp, synthetic construct
  source 1..22: mol_type = other DNA
caatactctcggcgatagagac

SEQ ID NO: 27 - protein, 673 aa, Xanthophyllomyces dendrorhous
MTALAYYQIHLIYTLPILGLLGLLTSPILTKFDIYKISILVFIAFSATTPWDSWIIRNGAWTYPSAESGQGVFGTFLDVPYEEYAFFVIQTVITGLVYVLATRHLLPSLALPKTRSSALSLALKALIPLPIIYLFTAHPSPSPDPLVTDHYFYMRALSLLITPPTMLLAALSGEYAFDWKSGRAKSTIAAIMIPTVYLIWVDYVAVGQDSWSINDEKIVGWRLGGVLPIEEAMFFLLTNLMIVLGLSACDHTQALYLLHGRTIYGNKKMPSSFPLITPPVLSLFFSSRPYSSQPKRDLELAVKLLEEKSRSFFVASAGFPSEVRERLVGLYAFCRVTDDLIDSPEVSSNPHATIDMVSDFLTLLFGPPLHPSQPDKILSSPLLPPSHPSRPTGMYPLPPPPSLSPAELVQFLTERVPVQYHFAFRLLAKLQGLIPRYPLDELLRGYTTDLIFPLSTEAVQARKTPIETTADLLDYGLCVAGSVAELLVYVSWASAPSQVPATIEEREAVLVASREMGTALQLVNIARDIKGDATEGRFYLPLSFFGLRDESKLAIPTDWTEPRPQDFDKLLSLSPSSTLPSSNASESFRFEWKTYSLPLVAYAEDLAKHSYKGIDRLPTEVQAGMRAACASYLLIGREIKVVWKGDVGERRTVAGWRRVRKVLSVVMSGWEGQ

SEQ ID NO: 28 - DNA, 2022 bp, Xanthophyllomyces dendrorhous
  source 1..2022: mol_type = genomic DNA
atgacggctctcgcatattaccagatccatctgatctatactctcccaattcttggtcttctcggcctgctcacttccccgattttgacaaaatttgacatctacaaaatatcgatcctcgtatttattgcgtttagtgcaaccacaccatgggactcatggatcatcagaaatggcgcatggacatatccatcagcggagagtggccaaggcgtgtttggaacgtttctagatgttccatatgaagagtacgctttctttgtcattcaaaccgtaatcaccggcttggtctacgtcttggcaactaggcaccttctcccatctctcgcgcttcccaagactagatcgtccgccctttctctcgcgctcaaggcgctcatccctctgcccattatctacctatttaccgctcaccccagcccatcgcccgacccgctcgtgacagatcactacttctacatgcgggcactctccttactcatcaccccacctaccatgctcttggcagcattatcaggcgaatatgctttcgattggaaaagtggccgagcaaagtcaactattgcagcaatcatgatcccgacggtgtatctgatttgggtagattatgttgctgtcggtcaagactcttggtcgatcaacgatgagaagattgtagggtggaggcttggaggtgtactacccattgaggaagctatgttcttcttactgacgaatctaatgattgttctgggtctgtctgcctgcgatcatactcaggccctatacctgctacacggtcgaactatttatggcaacaaaaagatgccatcttcatttcccctcattacaccgcctgtgctctccctgttttttagcagccgaccatactcttctcagccaaaacgtgacttggaactggcagtcaagttgttggaggaaaagagccggagcttttttgttgcctcggctggatttcctagcgaagttagggagaggctggttggactatacgcattctgccgggtgactgatgatcttatcgactctcctgaagtatcttccaacccgcatgccacaattgacatggtctccgattttcttaccctactatttgggcccccgctacacccttcgcaacctgacaagatcctttcttcgcctttacttcctccttcgcacccttcccgacccacgggaatgtatcccctcccgcctcctccttcgctctcgcctgccgagctcgttcaattccttaccgaaagggttcccgttcaataccatttcgccttcaggttgctcgctaagttgcaagggctgatccctcgatacccactcgacgaactccttagaggatacaccactgatcttatctttcccttatcgacagaggcagtccaggctcggaagacgcctatcgagaccacagctgacttgctggactatggtctatgtgtagcaggctcagtcgccgagctattggtctatgtctcttgggcaagtgcaccaagtcaggtccctgccaccatagaagaaagagaagctgtgttagtggcaagccgagagatgggaactgcccttcagttggtgaacattgctagggacattaaaggggacgcaacagaagggagattttacctaccactctcattctttggtcttcgggatgaatcaaagcttgcgatcccgactgattggacggaacctcggcctcaagatttcgacaaactcctcagtctatctccttcgtccacattaccatcttcaaacgcctcagaaagcttccggttcgaatggaagacgtactcgcttccattagtcgcctacgcagaggatcttgccaaacattcttataagggaattgaccgacttcctaccgaggttcaagcgggaatgcgagcggcttgcgcgagctacctactgatcggccgagagatcaaagtcgtttggaaaggagacgtcggagagagaaggacagttgccggatggaggagagtacggaaagtcttgagtgtggtcatgagcggatgggaagggcagtaa

SEQ ID NO: 29 - protein, 582 aa, Xanthophyllomyces dendrorhous
MGKEQDQDKPTAIIVGCGIGGIATAARLAKEGFQVTVFEKNDYSGGRCSLIERDGYRFDQGPSLLLLPDLFKQTFEDLGEKMEDWVDLIKCEPNYVCHFHDEETFTLSTDMALLKREVERFEGKDGFDRFLSFIQEAHRHYELAVVHVLQKNFPGFAAFLRLQFIGQILALHPFESIWTRVCRYFKTDRLRRVFSFAVMYMGQSPYSAPGTYSLLQYTELTEGIWYPRGGFWQVPNTLLQIVKRNNPSAKFNFNAPVSQVLLSPAKDRATGVRLESGEEHHADVVIVNADLVYASEHLIPDDARNKIGQLGEVKRSWWADLVGGKKLKGSCSSLSFYWSMDRIVDGLGGHNIFLAEDFKGSFDTIFEELGLPADPSFYVNVPSRIDPSAAPEGKDAIVILVPCGHIDASNPQDYNKLVARARKFVIHTLSAKLGLPDFEKMIVAEKVHDAPSWEKEFNLKDGSILGLAHNFMQVLGFRPSTRHPKYDKLFFVGASTHPGTGVPIVLAGAKLTANQVLESFDRSPAPDPNMSLSVPYGKPLKSNGTGIDSQVQLKFMDLERWVYLLVLLIGAVIARSVGVLAF

SEQ ID NO: 30 - DNA, 1749 bp, Xanthophyllomyces dendrorhous
  source 1..1749: mol_type = genomic DNA
atgggaaaagaacaagatcaggataaacccacagctatcatcgtgggatgtggtatcggtggaatcgccactgccgctcgtcttgctaaagaaggtttccaggtcacggtgttcgagaagaacgactactccggaggtcgatgctctttaatcgagcgagatggttatcgattcgatcaggggcccagtttgctgctcttgccagatctcttcaagcagacattcgaagatttgggagagaagatggaagattgggtcgatctcatcaagtgtgaacccaactatgtttgccacttccacgatgaagagactttcactctttcaaccgacatggcgttgctcaagcgggaagtcgagcgttttgaaggcaaagatggatttgatcggttcttgtcgtttatccaagaagcccacagacattacgagcttgctgtcgttcacgtcctgcagaagaacttccctggcttcgcagcattcttacggctacagttcattggccaaatcctggctcttcaccccttcgagtctatctggacaagagtttgtcgatatttcaagaccgacagattacgaagagtcttctcgtttgcagtgatgtacatgggtcaaagcccatacagtgcgcccggaacatattccttgctccaatacaccgaattgaccgagggcatctggtatccgagaggaggcttttggcaggttcctaatactcttcttcagatcgtcaagcgcaacaatccctcagccaagttcaatttcaacgctccagtttcccaggttcttctctctcctgccaaggaccgagcgactggtgttcgacttgaatccggcgaggaacatcacgccgatgttgtgattgtcaatgctgacctcgtttacgcctccgagcacttgattcctgacgatgccagaaacaagattggccaactgggtgaagtcaagagaagttggtgggctgacttagttggtggaaagaagctcaagggaagttgcagtagtttgagcttctactggagcatggaccgaatcgtggacggtctgggcggacacaatatcttcttggccgaggacttcaagggatcattcgacacaatcttcgaggagttgggtctcccagccgatccttccttttacgtgaacgttccctcgcgaatcgatccttctgccgctcccgaaggcaaagatgctatcgtcattcttgtgccgtgtggccatatcgacgcttcgaaccctcaagattacaacaagcttgttgctcgggcaaggaagtttgtgatccacacgctttccgccaagcttggacttcccgactttgaaaaaatgattgtggcagagaaggttcacgatgctccctcttgggagaaagaattcaacctcaaggacggaagcatcttgggactggctcacaactttatgcaagttcttggtttcaggccgagcaccagacatcccaagtatgacaagttgttctttgtcggggcttcgactcatcccggaactggggttcccatcgtcttggctggagccaagttaactgccaaccaagttctcgaatcctttgaccgatccccagctccagatcccaatatgtcactctccgtaccatatggaaaacctctcaaatcaaatggaacgggtatcgattctcaggtccagctgaagttcatggatttggagagatgggtataccttttggtgttgttgattggggccgtgatcgctcgatccgttggtgttcttgctttctga

SEQ ID NO: 31 - protein, 275 aa, Uncultured marine bacterium 66A03 [sequence omitted]

SEQ ID NO: 32 - DNA, 828 bp, Uncultured marine bacterium 66A03
  source 1..828: mol_type = genomic DNA
atgggcctgatgctgatcgactggtgtgccctggccctggtggtgttcatcggcctgccccacggcgccctggacgccgccatctctttctctatgatctcttctgccaagcgaatcgcccgactggccggcatcctgctgatctacctgctgctggccaccgccttcttcctgatctggtaccagctgcccgccttctctctgctgatcttcctgctgatctctatcatccacttcggcatggccgacttcaacgcctctccctctaagctgaagtggccccacatcatcgcccacggcggcgtggtgaccgtgtggctgcccctgatccagaagaacgaggtgaccaagctgttctctatcctgaccaacggccccacccccatcctgtgggacatcctgctgatcttcttcctgtgttggtctatcggcgtgtgtctgcacacctacgagaccctgcgatctaagcactacaacatcgccttcgagctgatcggcctgatcttcctggcctggtacgccccccccctggtgaccttcgccacctacttctgtttcatccactctcgacgacacttctctttcgtgtggaagcagctgcagcacatgtcttctaagaagatgatgatcggctctgccatcatcctgtcttgtacctcttggctgatcggcggcggcatctacttcttcctgaactctaagatgatcgcctctgaggccgccctgcagaccgtgttcatcggcctggccgccctgaccgtgccccacatgatcctgatcgacttcatcttccgaccccactcttctcgaatcaagatcaagaactag

SEQ ID NO: 33 - protein, 1508 aa, Yarrowia lipolytica
MDNGPIDPNRDVEQEHPVQVDHTEKHESSSSGAPLTQMSETSEDNTYTATPVPLTDVENMDPDSRDVNDLQRVLSNPESLHKLQSYTEQISRRMTQDERESLKNNEDTFDLARILDGFVQKSHEQGVHMRSAGVGWRNLTTDGIDQSTVFVPSVDELLRALATLPVQIAKAFKKKQTRHIIQNNNGVLKAGEMCLVLGRPGSGCSTFLKTITGQVGGYTGVEGDISYDGLSQKDMLEYFKSDIIYNGELDVHFPHLTVEETLNFAVGCRTPRQRLDGLTRDQYIKNYVQLLATVFGLRHTYNTKVGNDFVRGVSGGERKRVSIAEALATRASIFAWDNATRGLDASTALEYSQAIRATTNILNNASFVAIYQAGEHIYNLFDKVTVLYSGRQIYYGPADHAKDYFQRMGYECPPRQTTAEFLTAVTDPLGREPYPEMVGKVPTTADEFEKYWLASPEFRVVQAEYDDYVGSHNAEETFQNMQDSLSKDKMKRQRKKSPYLISFAMQMRLLTQRGFERLKGDMAYQTINVCANIIQALVIGSLFYNITESTAGAFSRGGVLFFTLLFNALASMAEISHSFSQRPIIVKQKSYSFYHPAGEALQALLTDIPGKLVTMICFTLIVYFLTHLNRTAGQFFAHLFILFVTTQCMTAFFQVLASATPSVEVANSLAGIGILIIVVYSGYMIPTPTMHVWFKWLNRANPVAYGFEALMANEFHNRVMTCEQIVPAGPDYSGMPESNKVCSFSGSTPGSLVVTGDNYIKNSYNYSFSHMWRNLGILFAFWMGFVFFNVTFSEYIQYHSSSGDVLLFKRGHIPEELQKEGADIDEVIADKAQADDSEKKMDRLLSLDEERDVFTWQNVDYVIPIAGGTRKLLDNVQGYVKPGTITALMGESGAGKTTLLNVLSQRINFGVITGDMLVNGRPLDRTFQRRTGYVQQQDLHLAESTVRESLIFSARLRQPSFVPDQEKIDYCDKIIKLLGMEAYAESLVGETGRGLNVEQRKKLSIGVELVAKPSLLLFLDEPTSGLDSQSAWAIVQFLKNLAAAGQAILCTIHQPSATLFEEFDRLLLLKKGGQTVYFGDIGKNSNTLVSYFERQGGRKCAPDENPAEYILECIGAGATATADGDWHDKWKNSEEYRQTTDEIAKLQQELAQRPQKELDPSLQRKYAAPYMTQLRWVLRRTQIQFWRSPGYIMAKFMLLIVGGLFIGFSFWDIKFTLSGMQNAIFAVFMITTLSVPLINQIQSFAFQSRELFEVRESSSNTFHWSCLLFSQFISELPYALIGGTIFYCCVYFPTKLGTSARVAGYFYFIYAILFNLYYLSFGLWILYFSPDVPSASIITSLMFSFVIAFCGVMQPASLMPGFWTFMYKLSPFTYIIQAYVGDVMHDRKITCLPREFSRFNPPSGQTCQEYAGKFLSQATGYLEDPNATTQCGYCPYSVADEFIATVGIKYHYRWRNVGFICAYIIFNICAMVLCYYLARVRVWRTGAAIADWKAKRANKKKAASSEKA

SEQ ID NO: 34 - DNA, 4527 bp, Yarrowia lipolytica
  source 1..4527: mol_type = genomic DNA
atggacaacggccctatcgatcccaatcgggacgtggagcaagaacacccggtgcaagtcgaccacaccgagaagcacgaatcttcctcctccggagctcctctaacgcagatgtcggaaacctcggaagataacacttacacggcgaccccggtgcctctcaccgatgtcgagaacatggaccccgattcccgggacgtgaacgatctgcagcgggtgctgtccaaccccgagtcgctgcacaagctgcagtcatacacagagcagatttctcgtcgaatgacccaagatgagcgagagtctctcaagaacaacgaagacacctttgacctggcccgaattctcgacggctttgtgcaaaagtcccacgagcaaggcgtgcacatgcgttctgcaggcgtgggctggagaaacctgaccaccgacggtatcgaccagtccaccgtctttgttccttcggtcgacgagctgctgcgagccctggccaccctgccagtccaaatcgctaaggctttcaagaagaagcagactcgacacattatccagaacaacaacggagtgctcaaggccggagagatgtgcctggtgctcggccgacctggatctggatgctccaccttcctcaagaccattaccggacaggtcggaggctacactggcgtggagggagacatttcatacgacggtctcagccagaaggacatgctggagtactttaagtcggacattatctacaatggagagctggacgtgcatttcccccatctcaccgtcgaagagactcttaactttgctgtcggatgccgaaccccacgacagcgtctggacggactcactcgagaccagtacatcaaaaactacgtccagctgctggcaaccgtcttcggtctgcgtcacacctacaacaccaaggttggaaacgatttcgttcgaggtgtgtctggaggagagcgaaagcgagtctctattgcagaggccctggctacccgagcttccatttttgcttgggataacgctactcgaggtctcgatgcctccactgctctggaatactctcaggccatccgagccaccactaacattctcaacaatgcgtcgtttgttgccatctaccaggccggagagcacatctacaacctctttgacaaggtcactgtgctctactctggtcgacagatttactacggacccgccgatcacgccaaggactacttccagcgaatgggttacgagtgccctcctcgacagactaccgccgagttcctcacagctgttaccgacccccttggccgagagccctaccctgagatggtcggcaaggtgcccaccaccgctgacgagttcgagaagtactggctggcctcccccgagttccgagtggtccaagccgagtacgacgactatgtgggttcccataacgccgaggagacattccagaacatgcaggactcgctgtccaaggataagatgaagcgacagcgaaagaagtcgccctacctcatctcctttgccatgcagatgcgactcctcacccagcgaggtttcgagcgtctcaagggagacatggcctaccagaccatcaacgtgtgtgccaacatcatccaggccctcgtcattggttcgcttttctacaacattactgagtccaccgctggagcattctctcgaggtggtgttcttttctttactcttctgtttaatgctctcgcctctatggccgagatttcccactccttctcccagcgacctattattgtgaagcaaaaaagttactcgttctaccaccctgccggcgaggccctccaggccctgctgaccgatatccccggtaagcttgttaccatgatctgtttcaccctcattgtttatttcttgacccacctgaaccgaacggccggccagttctttgcccatctgttcattttgttcgtcacaacccagtgtatgacggcctttttccaagtgctggcctctgccactccttccgttgaagttgccaattcgctggctggtattggtattctgattatcgtcgtctactctggttatatgatccccacccctaccatgcatgtgtggttcaagtggctgaaccgagccaaccctgtggcttacggtttcgaggccctgatggccaacgagtttcacaaccgagtcatgacctgtgagcagattgtgcccgctggtccagactactccggcatgcccgaatccaacaaggtctgctccttctctggttccacacccggttctctggtcgtcactggtgacaactacatcaagaactcgtacaactactctttctcgcacatgtggagaaacctgggtattctgtttgctttctggatgggcttcgttttcttcaacgtcaccttctccgagtacatccaataccactcctcttctggtgacgttctgctgtttaagcgaggccatattcccgaggagctgcagaaggagggtgctgatattgacgaggtgattgctgacaaggcccaggctgacgattccgagaagaagatggaccgcctcctctccctcgatgaagagcgagacgtcttcacctggcaaaatgtcgactatgtcattcctattgctggcggtactcgaaagctgctagataacgtgcagggttacgtcaagcccggtactatcactgctcttatgggagagtctggtgctggtaagaccactctactcaacgttctgtctcagcgaatcaactttggtgtcatcactggtgacatgcttgtcaacggccgacctctggatcgaactttccagcgacgaaccggttatgtccagcagcaggatctgcatcttgctgagtccactgttcgtgaatctctgattttctctgcccgtcttcgacagccctcttttgtccccgaccaggagaagattgactactgtgacaagatcatcaagctgcttggtatggaagcttacgcagagtctcttgttggagagactggtcgaggtctcaacgtggagcaacgaaagaagctgtctatcggtgtcgagcttgtcgccaagccttctttgctgctgttcttggatgagcctacttctggtcttgactctcagtctgcttgggctattgtccagttcctcaagaaccttgctgctgccggccaggccattctgtgtaccatccatcagccttctgctactctgtttgaggagtttgaccgtcttctgcttctgaagaagggtggccagaccgtctacttcggtgatattggtaagaactccaacaccctcgtctcttactttgagcgacagggtggtcgaaagtgtgctcccgatgagaaccctgccgaatacattctcgagtgtatcggtgccggtgctactgctactgccgatggagactggcacgataagtggaagaactctgaggagtaccgacagaccaccgatgagattgccaagctccaacaggagcttgctcagcgaccccagaaggaactggacccctctcttcagcgaaagtacgctgctccttacatgactcagctgcgatgggttcttcgacgaacccagattcagttctggcggtctcccggctacattatggccaagttcatgcttcttatcgttggtggtctcttcattggtttctctttttgggacatcaagttcaccctgtctggaatgcagaatgccattttcgctgtcttcatgatcaccactctgtctgtgcctcttatcaaccagatccagtcgtttgccttccagtcccgagagttgtttgaggttcgagagtcgtcgtccaacaccttccactggtcttgtctgctcttctctcagttcatttctgagctgccttacgctctgattggtggaaccatcttttactgctgtgtctacttccccaccaagctaggtacttctgctcgagtggccggatacttctacttcatctacgccattctgttcaacctgtactacctgtccttcggtctgtggattctctacttttcgcctgatgtgccctcggcttccatcattacctcgctcatgttctccttcgtcattgccttctgtggtgttatgcaacccgcttctctcatgcctggtttctggaccttcatgtacaagctgtctcccttcacctacattattcaggcctatgttggagatgttatgcatgaccgaaagattacctgtctgccccgagagttctctcgattcaaccctcccagtgggcagacttgtcaggagtatgctggtaagttcctgagccaggccaccggctaccttgaggaccccaacgccactacccagtgtggttactgcccttactctgtggctgacgagttcattgccactgtgggcatcaagtaccactaccgatggcgaaacgttggtttcatctgcgcctacatcatcttcaacatctgtgccatggttctttgctactacctggcccgtgttcgagtgtggcgaactggtgctgccattgctgactggaaggctaagcgagccaacaagaagaaggctgcttccagcgagaaggcctag

SEQ ID NO: 35 - DNA, 30 bp, synthetic construct
  source 1..30: mol_type = other DNA
attctcatcaggtagagccacccaccttgg

SEQ ID NO: 36 - DNA, 44 bp, synthetic construct
  source 1..44: mol_type = other DNA
atgcgccgccaacccggtctctggtgcttggagtggtgatatgt

SEQ ID NO: 37 - DNA, 44 bp, synthetic construct
  source 1..44: mol_type = other DNA
acatatcaccactccaagcaccagagaccgggttggcggcgcat

SEQ ID NO: 38 - DNA, 44 bp, synthetic construct
  source 1..44: mol_type = other DNA
atgacgagtcagacaggaggcatttgaatgattcttatactcag

SEQ ID NO: 39 - DNA, 44 bp, synthetic construct
  source 1..44: mol_type = other DNA
ctgagtataagaatcattcaaatgcctcctgtctgactcgtcat

SEQ ID NO: 40 - DNA, 44 bp, synthetic construct
  source 1..44: mol_type = other DNA
atgcgccgccaacccggtctcttggtggtattgtgactggggat

SEQ ID NO: 41 - DNA, 44 bp, synthetic construct
  source 1..44: mol_type = other DNA
atccccagtcacaataccaccaagagaccgggttggcggcgcat

SEQ ID NO: 42 - DNA, 44 bp, synthetic construct
  source 1..44: mol_type = other DNA
gatcgatagggccgttgtccattttgaatgattcttatactcag

SEQ ID NO: 43 - DNA, 44 bp, synthetic construct
  source 1..44: mol_type = other DNA
ctgagtataagaatcattcaaaatggacaacggccctatcgatc

SEQ ID NO: 44 - DNA, 30 bp, synthetic construct
  source 1..30: mol_type = other DNA
aaatggaagctcgggtagccagggcctctg

SEQ ID NO: 45 - DNA, 24 bp, synthetic construct
  source 1..24: mol_type = other DNA
gatcgggtcggaaagtgagataaa

SEQ ID NO: 46 - DNA, 24 bp, synthetic construct
  source 1..24: mol_type = other DNA
tgggtgttgaagacgccaatgttc